European Patent Application EP 4 218 408 A1, published August 2, 2023. Title: NON-HUMAN ANIMALS EXPRESSING EXOGENOUS TERMINAL DEOXYNUCLEOTIDYLTRANSFERASE. Applicant: REGENERON PHARMACEUTICALS, INC. Application EP EP23151094.2, filed June 2, 2017. The sequence listing filed with the application follows.

SEQUENCE LISTING (25 sequences)

SEQ ID NO: 1 - DNA, 13 bp, synthetic construct
  source 1..13: mol_type = other DNA
gtcgggtcgtggt

SEQ ID NO: 2-3 - skipped (2 entries)

SEQ ID NO: 4 - DNA, 99 bp, synthetic construct
  source 1..99: mol_type = other DNA
tattgcgtttttttaatcctttcagataaaagacctattcacaatcaaaaatggatccaccacgagcgtcccacttgagccctcggaagaagagacccc

SEQ ID NO: 5 - DNA, 108 bp, synthetic construct
  source 1..108: mol_type = other DNA
gccctggctgagggaaattttggaactcccaggctccagacccattctttgcgatcgctttagcaaaagcccctcagactcaggtatattgctctctgaatctacttt

SEQ ID NO: 6 - DNA, 107 bp, synthetic construct
  source 1..107: mol_type = other DNA
ccaaaggaaaacacattggcaaataccaacttctatgtggagatcctatggccggccggggatccagacatgataagatacattgatgagtttggacaaaccacaac

SEQ ID NO: 7 - DNA, 100 bp, synthetic construct
  source 1..100: mol_type = other DNA
tcgaccaggatgggcaccaccccggtgaacagctcctcgcccttgctcaccatgttggctaagctacctgggaacaatgggggggggggggggagtcaag

SEQ ID NO: 8 - DNA, 139 bp, synthetic construct
  source 1..139: mol_type = other DNA
catccttacatctttgtcatcccctgtatcaacatggaaaggcattaatgatctatgtcgggtgcggagaaagaggtaatgaaatggcaaccggtataacttcgtataatgtatgctatacgaagttatatgcatggcc

SEQ ID NO: 9 - DNA, 100 bp, synthetic construct
  source 1..100: mol_type = other DNA
ttcgtataatgtatgctatacgaagttatgtcgacctcgagggggggcccacctccagctgccttacagaaaagcaaatgcttgcttgcaacaatcacct

SEQ ID NO: 10 - DNA, 99 bp, synthetic construct; identical to SEQ ID NO: 4
  source 1..99: mol_type = other DNA

SEQ ID NO: 11 - DNA, 108 bp, synthetic construct; identical to SEQ ID NO: 5
  source 1..108: mol_type = other DNA

SEQ ID NO: 12 - DNA, 108 bp, synthetic construct
  source 1..108: mol_type = other DNA
cccaaaggaaaacacattggcaaataccaacttctatgtggagatcctatggccggccggggatccagacatgataagatacattgatgagtttggacaaaccacaac

SEQ ID NO: 13 - DNA, 100 bp, synthetic construct; identical to SEQ ID NO: 7
  source 1..100: mol_type = other DNA

SEQ ID NO: 14 - DNA, 151 bp, synthetic construct
  source 1..151: mol_type = other DNA
acctctgctgtgtctgcaagtttggcttgttcctgcttctgatttttgggtctagacccccgggctcgataactataacggtcctaaggtagcgactcgagcataaccactttcctgctatggatctgttaaatatccgccaaaggccaag

SEQ ID NO: 15 - DNA, 126 bp, synthetic construct
  source 1..126: mol_type = other DNA
catccttacatctttgtcatcccctgtatcaacatggaaaggcattaatgtcgctaccttaggaccgttatagttaggccccccctcgaggtcgacataacttcgtatagcatacattatacgaag

SEQ ID NO: 16 - DNA, 100 bp, synthetic construct
  source 1..100: mol_type = other DNA
ggccatgcatataacttcgtatagcatacattatacgaagttataccggtaaagaatgggtctggagcctgggagttccaaaatttccctcagccagggc

SEQ ID NO: 17 - DNA, 100 bp, synthetic construct
  source 1..100: mol_type = other DNA
cggggtctcttcttccgagggctcaagtgggacgctcgtggtggatccatggtgaggtcctgtgtgctcagtaactgtaaagagaacagtgatctcatgt

SEQ ID NO: 18 - DNA, 146 bp, synthetic construct
  source 1..146: mol_type = other DNA
tagtttccccaaacttaagtttatcgacttctaaaatgtatttagaattctgccatttcattacctctttctccgcacccgacatagataaagcttcataaccactttcctgctatggatctgttaaatatccgccaaaggccaag

SEQ ID NO: 19 - DNA, 22 bp, synthetic construct
  source 1..22: mol_type = other DNA
aagaagcacacgactgaggcac

SEQ ID NO: 20 - DNA, 55 bp, synthetic construct
  source 1..55: mol_type = other DNA
acactctttccctacacgacgctcttccgatctggaagatggatacagttggtgc

SEQ ID NO: 21 - DNA, 57 bp, synthetic construct
  source 1..57: mol_type = other DNA
gtgactggagttcagacgtgtgctcttccgatctaagcagtggtatcaacgcagagt

SEQ ID NO: 22 - DNA, 68 bp, synthetic construct
  source 1..68: mol_type = other DNA
aatgatacggcgaccaccgagatctacacnnnnnnacactctttccctacacgacgctcttccgatct

SEQ ID NO: 23 - DNA, 64 bp, synthetic construct
  source 1..64: mol_type = other DNA
caagcagaagacggcatacgagatnnnnnngtgactggagttcagacgtgtgctcttccgatct

SEQ ID NO: 24 - DNA, 24 bp, synthetic construct
  source 1..24: mol_type = other DNA
caccagtgtggccttgttagtctc

SEQ ID NO: 25 - DNA, 57 bp, synthetic construct
  source 1..57: mol_type = other DNA
acactctttccctacacgacgctcttccgatctaaggtggaaacagggtgactgatg